European Patent Application EP 4 810 069 A1, published September 23, 2026. Title: Imagining agents for GPC3. Applicant: Bayer Aktiengesellschaft. Application EP. The sequence listing filed with the application follows.

SEQUENCE LISTING (42 sequences)

SEQ ID NO: 1 - protein, 115 aa, synthetic construct
QVQLVQSGAEVKKPGASVKVSCKASGYTFTDYEMHWVRQAPGQGLEWMGALDPKTGDTAYSQKFKGRVTLTADKSTSTAYMELSSLTSEDTAVYYCTRFYSYTYWGQGTLVTVSS

SEQ ID NO: 2 - protein, 5 aa, synthetic construct
DYEMH

SEQ ID NO: 3 - protein, 17 aa, synthetic construct
ALDPKTGDTAYSQKFKG

SEQ ID NO: 4 - protein, 6 aa, synthetic construct
FYSYTY

SEQ ID NO: 5 - protein, 112 aa, synthetic construct
DVVMTQSPLSLPVTPGEPASISCRSSQSLVHSNRNTYLHWYLQKPGQSPQLLIYKVSNRFSGVPDRFSGSGSGTDFTLKISRVEAEDVGVYYCSQNTHVPPTFGQGTKLEIK

SEQ ID NO: 6 - protein, 16 aa, synthetic construct
RSSQSLVHSNRNTYLH

SEQ ID NO: 7 - protein, 7 aa, synthetic construct
KVSNRFS

SEQ ID NO: 8 - protein, 9 aa, synthetic construct
SQNTHVPPT

SEQ ID NO: 9 - protein, 445 aa, synthetic construct
QVQLVQSGAEVKKPGASVKVSCKASGYTFTDYEMHWVRQAPGQGLEWMGALDPKTGDTAYSQKFKGRVTLTADKSTSTAYMELSSLTSEDTAVYYCTRFYSYTYWGQGTLVTVSSASTKGPSVFPLAPSSKSTSGGTAALGCLVKDYFPEPVTVSWNSGALTSGVHTFPAVLQSSGLYSLSSVVTVPSSSLGTQTYICNVNHKPSNTKVDKKVEPKSCDKTHTCPPCPAPELLGGPSVFLFPPKPKDTLMISRTPEVTCVVVDVSHEDPEVKFNWYVDGVEVHNAKTKPREEQYNSTYRVVSVLTVLHQDWLNGKEYKCKVSNKALPAPIEKTISKAKGQPREPQVYTLPPSRDELTKNQVSLTCLVKGFYPSDIAVEWESNGQPENNYKTTPPVLDSDGSFFLYSKLTVDKSRWQQGNVFSCSVMHEALHNHYTQKSLSLSPGK

SEQ ID NO: 10 - protein, 219 aa, synthetic construct
DVVMTQSPLSLPVTPGEPASISCRSSQSLVHSNRNTYLHWYLQKPGQSPQLLIYKVSNRFSGVPDRFSGSGSGTDFTLKISRVEAEDVGVYYCSQNTHVPPTFGQGTKLEIKRTVAAPSVFIFPPSDEQLKSGTASVVCLLNNFYPREAKVQWKVDNALQSGNSQESVTEQDSKDSTYSLSSTLTLSKADYEKHKVYACEVTHQGLSSPVTKSFNRGEC

SEQ ID NO: 11 - protein, 115 aa, synthetic construct
QVQLVQSGAEVKKPGASVKVSCKASGYTFTDYEMHWVRQAPGQGLEWMGALDPSTGSTSYAQRFQGRVTMTRDTSTSTVYMELSSLRSEDTAVYYCTRFYSYTYWGQGTLVTVSS

SEQ ID NO: 12 - protein, 5 aa, synthetic construct
DYEMH

SEQ ID NO: 13 - protein, 17 aa, synthetic construct
ALDPSTGSTSYAQRFQG

SEQ ID NO: 14 - protein, 6 aa, synthetic construct
FYSYTY

SEQ ID NO: 15 - protein, 112 aa, synthetic construct
DIVMTQSPLSLPVTPGEPASISCRSSQSLLHSNGYNYLHWYLQKPGQSPQLLIYRGSNRASGVPDRFSGSGSGTDFTLKISRVEAEDVGVYYCSQNTHVPYTFGQGTKLEIK

SEQ ID NO: 16 - protein, 16 aa, synthetic construct
RSSQSLLHSNGYNYLH

SEQ ID NO: 17 - protein, 7 aa, synthetic construct
RGSNRAS

SEQ ID NO: 18 - protein, 9 aa, synthetic construct
SQNTHVPYT

SEQ ID NO: 19 - DNA, 345 bp, synthetic construct
  source 1..345: mol_type = other DNA
caggttcagctggttcagtctggcgccgaagtgaagaaacctggcgcctctgtgaaggtgtcctgcaaggccagcggctacacctttaccgactacgagatgcactgggtccgacaggctccaggacaaggcttggaatggatgggagccctggatcctagcaccggcagcacatcttacgcccagagattccagggcagagtgaccatgaccagagacaccagcacctccaccgtgtacatggaactgagcagcctgagaagcgaggacaccgccgtgtactactgcacccggttctacagctacacctactggggccagggcaccctggtcacagtttcttca

SEQ ID NO: 20 - DNA, 15 bp, synthetic construct
  source 1..15: mol_type = other DNA
gactacgagatgcac

SEQ ID NO: 21 - DNA, 51 bp, synthetic construct
  source 1..51: mol_type = other DNA
gccctggatcctagcaccggcagcacatcttacgcccagagattccagggc

SEQ ID NO: 22 - DNA, 18 bp, synthetic construct
  source 1..18: mol_type = other DNA
ttctacagctacacctac

SEQ ID NO: 23 - DNA, 336 bp, synthetic construct
  source 1..336: mol_type = other DNA
gacatcgtgatgacacagagccctctgagcctgcctgtgacacctggcgaacctgccagcatcagctgtagaagcagccagtctctgctgcacagcaacggctacaactacctgcactggtatctgcagaagcccggccagtctcctcagctgctgatctacagaggcagcaacagagccagcggcgtgcccgatagattttctggctctggcagcggcaccgacttcaccctgaagatctctagagtggaagccgaggacgtgggcgtgtactactgcagccagaatacccacgtgccatacacctttggccagggcaccaagctggaaatcaaa

SEQ ID NO: 24 - DNA, 48 bp, synthetic construct
  source 1..48: mol_type = other DNA
agaagcagccagtctctgctgcacagcaacggctacaactacctgcac

SEQ ID NO: 25 - DNA, 21 bp, synthetic construct
  source 1..21: mol_type = other DNA
agaggcagcaacagagccagc

SEQ ID NO: 26 - DNA, 27 bp, synthetic construct
  source 1..27: mol_type = other DNA
agccagaatacccacgtgccatacacc

SEQ ID NO: 27 - protein, 445 aa, synthetic construct
QVQLVQSGAEVKKPGASVKVSCKASGYTFTDYEMHWVRQAPGQGLEWMGALDPSTGSTSYAQRFQGRVTMTRDTSTSTVYMELSSLRSEDTAVYYCTRFYSYTYWGQGTLVTVSSASTKGPSVFPLAPSSKSTSGGTAALGCLVKDYFPEPVTVSWNSGALTSGVHTFPAVLQSSGLYSLSSVVTVPSSSLGTQTYICNVNHKPSNTKVDKKVEPKSCDKTHTCPPCPAPELLGGPSVFLFPPKPKDTLMISRTPEVTCVVVDVSHEDPEVKFNWYVDGVEVHNAKTKPREEQYNSTYRVVSVLTVLHQDWLNGKEYKCKVSNKALPAPIEKTISKAKGQPREPQVYTLPPSRDELTKNQVSLTCLVKGFYPSDIAVEWESNGQPENNYKTTPPVLDSDGSFFLYSKLTVDKSRWQQGNVFSCSVMHEALHNHYTQKSLSLSPGK

SEQ ID NO: 28 - protein, 219 aa, synthetic construct
DIVMTQSPLSLPVTPGEPASISCRSSQSLLHSNGYNYLHWYLQKPGQSPQLLIYRGSNRASGVPDRFSGSGSGTDFTLKISRVEAEDVGVYYCSQNTHVPYTFGQGTKLEIKRTVAAPSVFIFPPSDEQLKSGTASVVCLLNNFYPREAKVQWKVDNALQSGNSQESVTEQDSKDSTYSLSSTLTLSKADYEKHKVYACEVTHQGLSSPVTKSFNRGEC

SEQ ID NO: 29 - DNA, 1335 bp, synthetic construct
  source 1..1335: mol_type = other DNA
caggttcagctggttcagtctggcgccgaagtgaagaaacctggcgcctctgtgaaggtgtcctgcaaggccagcggctacacctttaccgactacgagatgcactgggtccgacaggctccaggacaaggcttggaatggatgggagccctggatcctagcaccggcagcacatcttacgcccagagattccagggcagagtgaccatgaccagagacaccagcacctccaccgtgtacatggaactgagcagcctgagaagcgaggacaccgccgtgtactactgcacccggttctacagctacacctactggggccagggcaccctggtcacagtttcttcagccagcaccaagggccccagcgtgttccctctggcccctagcagcaagagcacatctggcggaacagccgccctgggctgcctcgtgaaggactactttcccgagcccgtgaccgtgtcctggaactctggcgctctgacaagcggcgtgcacacctttccagccgtgctgcagagcagcggcctgtactctctgagcagcgtcgtgacagtgcccagcagctctctgggcacccagacctacatctgcaacgtgaaccacaagcccagcaacaccaaggtggacaagaaggtggaacccaagagctgcgacaagacccacacctgtcccccttgtcctgcccccgaactgctgggaggcccttccgtgttcctgttccccccaaagcccaaggacaccctgatgatcagccggacccccgaagtgacctgcgtggtggtggatgtgtcccacgaggaccctgaagtgaagttcaattggtacgtggacggcgtggaagtgcacaacgccaagaccaagcctagagaggaacagtacaacagcacctaccgggtggtgtccgtgctgacagtgctgcaccaggactggctgaacggcaaagagtacaagtgcaaggtgtccaacaaggccctgcctgcccccatcgagaaaaccatcagcaaggccaagggccagccccgcgaaccccaggtgtacacactgcccccaagcagggacgagctgaccaagaaccaggtgtccctgacctgtctcgtgaaaggcttctacccctccgatatcgccgtggaatgggagagcaacggccagcccgagaacaactacaagaccaccccccctgtgctggacagcgacggctcattcttcctgtacagcaagctgaccgtggacaagtcccggtggcagcagggcaacgtgttcagctgcagcgtgatgcacgaggccctgcacaaccactacacccagaagtccctgagcctgagccctggcaag

SEQ ID NO: 30 - DNA, 657 bp, synthetic construct
  source 1..657: mol_type = other DNA
gacatcgtgatgacacagagccctctgagcctgcctgtgacacctggcgaacctgccagcatcagctgtagaagcagccagtctctgctgcacagcaacggctacaactacctgcactggtatctgcagaagcccggccagtctcctcagctgctgatctacagaggcagcaacagagccagcggcgtgcccgatagattttctggctctggcagcggcaccgacttcaccctgaagatctctagagtggaagccgaggacgtgggcgtgtactactgcagccagaatacccacgtgccatacacctttggccagggcaccaagctggaaatcaaacgaaccgtggccgctcccagcgtgttcatcttcccacctagcgacgagcagctgaagtccggcacagcctctgtcgtgtgcctgctgaacaacttctacccccgcgaggccaaggtgcagtggaaggtggacaatgccctgcagagcggcaacagccaggaaagcgtgaccgagcaggacagcaaggactccacctacagcctgagcagcaccctgaccctgagcaaggccgactacgagaagcacaaggtgtacgcctgcgaagtgacccaccagggcctgtctagccccgtgaccaagagcttcaaccggggcgagtgt

SEQ ID NO: 31 - protein, 135 aa, synthetic construct
QVQLVQSGGGLVQPGGSLRLSCAASYFDFDSYEMSWVRQAPGKGLEWIGSIYHSGSTYYNPSLKSRVTISRDNSKNTLYLQMNTLRAEDTATYYCARVNMDRFDYWGQGTLVTVSSSAGEQKLISEEDLHHHHHH

SEQ ID NO: 32 - protein, 222 aa, synthetic construct
QVQLVQSGAEVKKPGASVKVSCKASGYTFTDYEMHWVRQAPGQGLEWMGALDPSTGSTSYAQRFQGRVTMTRDTSTSTVYMELSSLRSEDTAVYYCTRFYSYTYWGQGTLVTVSSASTKGPSVFPLAPSSKSTSGGTAALGCLVKDYFPEPVTVSWNSGALTSGVHTFPAVLQSSGLYSLSSVVTVPSSSLGTQTYICNVNHKPSNTKVDKKVEPKSCDKTH

SEQ ID NO: 33 - protein, 219 aa, synthetic construct; identical to SEQ ID NO: 28

SEQ ID NO: 34 - protein, 226 aa, synthetic construct
EVQLLESGGGLVQPGGSLRLSCAASGFTFGDYAMSWVRQAPGKGLEWVSGISGSGGSTYYADSVKGRFTISRDNSKNTLYLQMNSLRAEDTAVYYCAREGETSFGLDVWGQGTLVTVSSASTKGPSVFPLAPSSKSTSGGTAALGCLVKDYFPEPVTVSWNSGALTSGVHTFPAVLQSSGLYSLSSVVTVPSSSLGTQTYICNVNHKPSNTKVDKKVEPKSCDKTH

SEQ ID NO: 35 - protein, 217 aa, synthetic construct
QSVLTQPPSASGTPGQRVTISCSGSSSNIGSNYVYWYQQLPGTAPKLLIYDNNDRPSGVPDRFSGSKSGTSASLAISGLRSEDEADYYCVAWDDSLNGHWVFGGGTKLTVLGQPKAAPSVTLFPPSSEELQANKATLVCLISDFYPGAVTVAWKADSSPVKAGVETTTPSKQSNNKYAASSYLSLTPEQWKSHRSYSCQVTHEGSTVEKTVAPTECS

SEQ ID NO: 36 - protein, 234 aa, synthetic construct
QVQLVQSGAEVKKPGASVKVSCKASGYTFTDYEMHWVRQAPGQGLEWMGALDPSTGSTSYAQRFQGRVTMTRDTSTSTVYMELSSLRSEDTAVYYCTRFYSYTYWGQGTLVTVSSASTKGPSVFPLAPSSKSTSGGTAALGCLVKDYFPEPVTVSWNSGALTSGVHTFPAVLQSSGLYSLSSVVTVPSSSLGTQTYICNVNHKPSNTKVDKKVEPKSCDKTHTCPPCPAPELLG

SEQ ID NO: 37 - protein, 218 aa, synthetic construct
IVMTQSPLSLPVTPGEPASISCRSSQSLLHSNGYNYLHWYLQKPGQSPQLLIYRGSNRASGVPDRFSGSGSGTDFTLKISRVEAEDVGVYYCSQNTHVPYTFGQGTKLEIKRTVAAPSVFIFPPSDEQLKSGTASVVCLLNNFYPREAKVQWKVDNALQSGNSQESVTEQDSKDSTYSLSSTLTLSKADYEKHKVYACEVTHQGLSSPVTKSFNRGEC

SEQ ID NO: 38 - protein, 238 aa, synthetic construct
EVQLLESGGGLVQPGGSLRLSCAASGFTFGDYAMSWVRQAPGKGLEWVSGISGSGGSTYYADSVKGRFTISRDNSKNTLYLQMNSLRAEDTAVYYCAREGETSFGLDVWGQGTLVTVSSASTKGPSVFPLAPSSKSTSGGTAALGCLVKDYFPEPVTVSWNSGALTSGVHTFPAVLQSSGLYSLSSVVTVPSSSLGTQTYICNVNHKPSNTKVDKKVEPKSCDKTHTCPPCPAPELLG

SEQ ID NO: 39 - protein, 217 aa, synthetic construct; identical to SEQ ID NO: 35

SEQ ID NO: 40 - protein, 271 aa, synthetic construct
QVQLVQSGAEVKKPGASVKVSCKASGYTFTDYEMHWVRQAPGQGLEWMGALDPKTGDTAYSQKFKGRVTLTADKSTSTAYMELSSLTSEDTAVYYCTRFYSYTYWGQGTLVTVSSGGGGSGGGGSGGGGSDVVMTQSPLSLPVTPGEPASISCRSSQSLVHSNRNTYLHWYLQKPGQSPQLLIYKVSNRFSGVPDRFSGSGSGTDFTLKISRVEAEDVGVYYCSQNTHVPPTFGQGTKLEIKGGGGSGGGGSGGGGSGVECPPCPAPELLG

SEQ ID NO: 41 - protein, 481 aa, synthetic construct
QVQLVQSGAEVKKPGASVKVSCKASGYTFTDYEMHWVRQAPGQGLEWMGALDPKTGDTAYSQKFKGRVTLTADKSTSTAYMELSSLTSEDTAVYYCTRFYSYTYWGQGTLVTVSSGGGGSGGGGSGGGGSDVVMTQSPLSLPVTPGEPASISCRSSQSLVHSNRNTYLHWYLQKPGQSPQLLIYKVSNRFSGVPDRFSGSGSGTDFTLKISRVEAEDVGVYYCSQNTHVPPTFGQGTKLEIKGGGGSGGGGSGGGGSGVECPPCPAPELLGGPSVFLFPPKPKDTLMISRTPEVTCVVVDVSHEDPEVKFNWYVDGVEVHNAKTKPREEQYNSTYRVVSVLTVLHQDWLNGKEYKCKVSNKALPAPIEKTISKAKGQPREPQVYTLPPSRDELTKNQVSLTCLVKGFYPSDIAVEWESNGQPENNYKTTPPVLDSDGSFFLYSKLTVDKSRWQQGNVFSCSVMHEALHNHYTQKSLSLSPG

SEQ ID NO: 42 - protein, 556 aa, Homo sapiens
QPPPPPPDATCHQVRSFFQRLQPGLKWVPETPVPGSDLQVCLPKGPTCCSRKMEEKYQLTARLNMEQLLQSASMELKFLIIQNAAVFQEAFEIVVRHAKNYTNAMFKNNYPSLTPQAFEFVGEFFTDVSLYILGSDINVDDMVNELFDSLFPVIYTQLMNPGLPDSALDINECLRGARRDLKVFGNFPKLIMTQVSKSLQVTRIFLQALNLGIEVINTTDHLKFSKDCGRMLTRMWYCSYCQGLMMVKPCGGYCNVVMQGCMAGVVEIDKYWREYILSLEELVNGMYRIYDMENVLLGLFSTIHDSIQYVQKNAGKLTTTIGKLCAHSQQRQYRSAYYPEDLFIDKKVLKVAHVEHEETLSSRRRELIQKLKSFISFYSALPGYICSHSPVAENDTLCWNGQELVERYSQKAARNGMKNQFNLHELKMKGPEPVVSQIIDKLKHINQLLRTMSMPKGRVLDKNLDEEGFESGDCGDDEDECIGGSGDGMIKVKNQLRFLAELAYDLDVDDAPGNSQQATPKDNEISTFHNLGNVHSPLKLLTSMAISVVCFFFLVH